European Patent Application EP 4 563 596 A1, published June 4, 2025. Title: ANTI-CD163 ANTIBODIES WITH IMPROVED ADCC CAPABILITIES. Applicant: OncoSpear ApS. Application EP. The sequence listing filed with the application follows.

SEQUENCE LISTING (26 sequences)

SEQ ID NO: 1 - protein, 243 aa, synthetic construct
MDMRVPAMDMRVPAQLLGLLLLWLPGARCDIVMTQSPSSLSASVGDRVTITCRASQSVSSDVAWFQQKPGKSPKPLIYYASNRYSGVPSRFSGSGSGTDFTLTISSLQAEDFAVYFCGQDYTSPRTFGGGTKLEIKRTVAAPSVFIFPPSDEQLKSGTASVVCLLNNFYPREAKVQWKVDNALQSGNSQESVTEQDSKDSTYSLSSTLTLSKADYEKHKVYACEVTHQGLSSPVTKSFNRGEC

SEQ ID NO: 2 - protein, 243 aa, synthetic construct
MDMRVPAMDMRVPAQLLGLLLLWLPGARCDIVMTQSPSSLSASVGDRVTITCRASQSVSSDVAWFQQKPGKSPKPLIYYASNRYSGVPSRFSGSGSGTDFTLTISSLQAEDFAVYFCQQDYTSPRTFGGGTKLEIKRTVAAPSVFIFPPSDEQLKSGTASVVCLLNNFYPREAKVQWKVDNALQSGNSQESVTEQDSKDSTYSLSSTLTLSKADYEKHKVYACEVTHQGLSSPVTKSFNRGEC

SEQ ID NO: 3 - protein, 458 aa, synthetic construct
MKHLWFFLLLVAAPRWVLSQVQLQESGPGLVKPSETLSLTCTVSGYSITSDYAWNWIRQFPGNKLEWMGYITYSGSTYYNPSLKSRVTISVDTSKNQFSLKLSSVTAADTATYYCVSGTYYFDYWGQGTTLTVSSASTKGPSVFPLAPCSRSTSESTAALGCLVKDYFPEPVTVSWNSGALTSGVHTFPAVLQSSGLYSLSSVVTVPSSSLGTKTYTCNVDHKPSNTKVDKRVESKYGPPCPSCPAPEFLGGPSVFLFPPKPKDTLMISRTPEVTCVVVDVSQEDPEVQFNWYVDGVEVHNAKTKPREEQFNSTYRVVSVLTVLHQDWLNGKEYKCKVSNKGLPSSIEKTISKAKGQPREPQVYTLPPSQEEMTKNQVSLTCLVKGFYPSDIAVEWESNGQPENNYKTTPPVLDSDGSFFLYSRLTVDKSRWQEGNVFSCSVMHEALHNHYTQKSLSL

SEQ ID NO: 4 - protein, 465 aa, synthetic construct
MKHLWFFLLLVAAPRWVLSQVQLQESGPGLVKPSETLSLTCTVSGYSITSDYAWNWIRQFPGNKLEWMGYITYSGSTYYNPSLKSRVTISVDTSKNQFSLKLSSVTAADTATYYCVSGTYYFDYWGQGTTLTVSSASTKGPSVFPLAPSSKSTSGGTAALGCLVKDYFPEPVTVSWNSGALTSGVHTFPAVLQSSGLYSLSSVVTVPSSSLGTQTYICNVNHKPSNTKVDKKVEPKSCDKTHTCPPCPAPELLGGPSVFLFPPKPKDTLMISRTPEVTCVVVDVSHEDPEVKFNWYVDGVEVHNAKTKPREEQYNSTYRVVSVLTVLHQDWLNGKEYKCKVSNKALPAPIEKTISKAKGQPREPQVYTLPPSRDELTKNQVSLTCLVKGFYPSDIAVEWESNGQPENNYKTTPPVLDSDGSFFLYSKLTVDKSRWQQGNVFSCSVMHEALHNHYTQKSLSLSPGK

SEQ ID NO: 5 - protein, 465 aa, synthetic construct
MKHLWFFLLLVAAPRWVLSQVQLQESGPGLVKPSETLSLTCTVSGYSITSDYAWNWIRQFPGNKLEWMGYITYSGSTYYNPSLKSRVTISVDTSKNQFSLKLSSVTAADTATYYCVSGTYYFDYWGQGTTLTVSSASTKGPSVFPLAPSSKSTSGGTAALGCLVKDYFPEPVTVSWNSGALTSGVHTFPAVLQSSGLYSLSSVVTVPSSSLGTQTYICNVNHKPSNTKVDKKVEPKSCDKTHTCPPCPAPELLGGPSVFLFPPKPKDTLMISRTPEVTCVVVDVSFEDPEVKFNWYVDGVEVHNAKTKPREEQYNSTYRVVSVLTVLHQDWLNGKEYKCKVTNKALPAPIEKTISKAKGQPREPQVYTLPPSRDELTKNQVSLTCLVKGFYPSDIAVEWESNGQPENNYKTTPPVLDSDGSFFLYSKLTVDKSRWQQGNVFSCSVMHEALHNHYTQKSLSLSPGK

SEQ ID NO: 6 - protein, 465 aa, synthetic construct
MKHLWFFLLLVAAPRWVLSQVQLQESGPGLVKPSETLSLTCTVSGYSITSDYAWNWIRQFPGNKLEWMGYITYSGSTYYNPSLKSRVTISVDTSKNQFSLKLSSVTAADTATYYCVSGTYYFDYWGQGTTLTVSSASTKGPSVFPLAPSSKSTSGGTAALGCLVKDYFPEPVTVSWNSGALTSGVHTFPAVLQSSGLYSLSSVVTVPSSSLGTQTYICNVNHKPSNTKVDKKVEPKSCDKTHTCPPCPAPELLGGPSVFLFPPKIKDTLMISRTPEVTCVVVDVSHEDPEVKFNWYVDGVEVHNAKTKPREEQYNSTYRVVSVLTVLHQDWLNGKEYKCKVSNKALPAPIEKTISKQKGQPREPQVYTLPPSRDELTKNQVSLTCLVKGFYPSDIAVEWESNGQPENNYKTTPPVLDSDGSFFLYSKLTVDKSRWQQGNVFSCSVMHEALHNHYTQKSLSLSPGK

SEQ ID NO: 7 - protein, 464 aa, synthetic construct
MKHLWFFLLLVAAPRWVLSQVQLQESGPGLVKPSETLSLTCTVSGYSITSDYAWNWIRQFPGNKLEWMGYITYSGSTYYNPSLKSRVTISVDTSKNQFSLKLSSVTAADTATYYCVSGTYYFDYWGQGTTLTVSSASTKGPSVFPLAPSSKSTSGGTAALGCLVKDYFPEPVTVSWNSGALTSGVHTFPAVLQSSGLYSLSSVVTVPSSSLGTQTYICNVNHKPSNTKVDKKVEPKSCDKTHTCPPCPAPELLGGPSVFLFPPKPKDTLMISRTPEVTCVVVDVSHEDPEVKFNWYVDGVEVHNAKTKPREEQYNYARVVSVLTVLHQDWLNGKEYKCKVSNKALPAPIAATISKAKGQPREPQVYTLPPSRDELTKNQVSLTCLVKGFYPSDIAVEWESNGQPENNYKTTPPVLDSDGSFFLYSKLTVDKSRWQQGNVFSCSVMHEALHNHYTQKSLSLSPGK

SEQ ID NO: 8 - protein, 465 aa, synthetic construct
MKHLWFFLLLVAAPRWVLSQVQLQESGPGLVKPSETLSLTCTVSGYSITSDYAWNWIRQFPGNKLEWMGYITYSGSTYYNPSLKSRVTISVDTSKNQFSLKLSSVTAADTATYYCVSGTYYFDYWGQGTTLTVSSASTKGPSVFPLAPSSKSTSGGTAALGCLVKDYFPEPVTVSWNSGALTSGVHTFPAVLQSSGLYSLSSVVTVPSSSLGTQTYICNVNHKPSNTKVDKKVEPKSCDKTHTCPPCPAPELVGGPSVFLLPPKPKDTLMISRTPEVTCVVVDVSHEDPEVKFNWYVDGVEVHNAKTKPPEEQYNSTLRVVSVLTVLHQDWLNGKEYKCKVSNKALPAPIEKTISKAKGQPREPQVYTLPPSRDELTKNQVSLTCLVKGFYPSDIAVEWESNGQPENNYKTTPLVLDSDGSFFLYSKLTVDKSRWQQGNVFSCSVMHEALHNHYTQKSLSLSPGK

SEQ ID NO: 9 - protein, 465 aa, synthetic construct
MKHLWFFLLLVAAPRWVLSQVQLQESGPGLVKPSETLSLTCTVSGYSITSDYAWNWIRQFPGNKLEWMGYITYSGSTYYNPSLKSRVTISVDTSKNQFSLKLSSVTAADTATYYCVSGTYYFDYWGQGTTLTVSSASTKGPSVFPLAPSSKSTSGGTAALGCLVKDYFPEPVTVSWNSGALTSGVHTFPAVLQSSGLYSLSSVVTVPSSSLGTQTYICNVNHKPSNTKVDKKVEPKSCDKTHTCPPCPAPELLGGPDVFLFPPKPKDTLMISRTPEVTCVVVDVSHEDPEVKFNWYVDGVEVHNAKTKPREEQYNSTYRVVSVLTVLHQDWLNGKEYKCKVSNKALPLPEEKTISKAKGQPREPQVYTLPPSRDELTKNQVSLTCLVKGFYPSDIAVEWESNGQPENNYKTTPPVLDSDGSFFLYSKLTVDKSRWQQGNVFSCSVMHEALHNHYTQKSLSLSPGK

SEQ ID NO: 10 - protein, 465 aa, synthetic construct
MKHLWFFLLLVAAPRWVLSQVQLQESGPGLVKPSETLSLTCTVSGYSITSDYAWNWIRQFPGNKLEWMGYITYSGSTYYNPSLKSRVTISVDTSKNQFSLKLSSVTAADTATYYCVSGTYYFDYWGQGTTLTVSSASTKGPSVFPLAPSSKSTSGGTAALGCLVKDYFPEPVTVSWNSGALTSGVHTFPAVLQSSGLYSLSSVVTVPSSSLGTQTYICNVNHKPSNTKVDKKVEPKSCDKTHTCPPCPAPELLAGPDVFLFPPKPKDTLMISRTPEVTCVVVDVSHEDPEVKFNWYVDGVEVHNAKTKPREEQYNSTYRVVSVLTVLHQDWLNGKEYKCKVSNKALPAPEEKTISKAKGQPREPQVYTLPPSRDELTKNQVSLTCLVKGFYPSDIAVEWESNGQPENNYKTTPPVLDSDGSFFLYSKLTVDKSRWQQGNVFSCSVMHEALHNHYTQKSLSLSPGK

SEQ ID NO: 11 - protein, 465 aa, synthetic construct
MKHLWFFLLLVAAPRWVLSQVQLQESGPGLVKPSETLSLTCTVSGYSITSDYAWNWIRQFPGNKLEWMGYITYSGSTYYNPSLKSRVTISVDTSKNQFSLKLSSVTAADTATYYCVSGTYYFDYWGQGTTLTVSSASTKGPSVFPLAPSSKSTSGGTAALGCLVKDYFPEPVTVSWNSGALTSGVHTFPAVLQSSGLYSLSSVVTVPSSSLGTQTYICNVNHKPSNTKVDKKVEPKSCDKTHTCPPCPAPELLAGPDVFLFPPKPKDTLMISRTPEVTCVVVDVSHEDPEVKFNWYVDGVEVHNAKTKPREEQYNSTYRVVSVLTVLHQDWLNGKEYKCKVSNKALPLPEEKTISKAKGQPREPQVYTLPPSRDELTKNQVSLTCLVKGFYPSDIAVEWESNGQPENNYKTTPPVLDSDGSFFLYSKLTVDKSRWQQGNVFSCSVMHEALHNHYTQKSLSLSPGK

SEQ ID NO: 12 - protein, 465 aa, synthetic construct
MKHLWFFLLLVAAPRWVLSQVQLQESGPGLVKPSETLSLTCTVSGYSITSDYAWNWIRQFPGNKLEWMGYITYSGSTYYNPSLKSRVTISVDTSKNQFSLKLSSVTAADTATYYCVSGTYYFDYWGQGTTLTVSSASTKGPSVFPLAPSSKSTSGGTAALGCLVKDYFPEPVTVSWNSGALTSGVHTFPAVLQSSGLYSLSSVVTVPSSSLGTQTYICNVNHKPSNTKVDKKVEPKSCDKTHTCPPCPAPELLGGPDVFLFPPKPKDTLMISRTPEVTCVVVDVSHEDPEVKFNWYVDGVEVHNAKTKPREEQYNSTYRVVSVLTVLHQDWLNGKEYKCKVSNKALPAPEEKTISKAKGQPREPQVYTLPPSRDELTKNQVSLTCLVKGFYPSDIAVEWESNGQPENNYKTTPPVLDSDGSFFLYSKLTVDKSRWQQGNVFSCSVMHEALHNHYTQKSLSLSPGK

SEQ ID NO: 13 - protein, 465 aa, synthetic construct
MKHLWFFLLLVAAPRWVLSQVQLQESGPGLVKPSETLSLTCTVSGYSITSDYAWNWIRQFPGNKLEWMGYITYSGSTYYNPSLKSRVTISVDTSKNQFSLKLSSVTAADTATYYCVSGTYYFDYWGQGTTLTVSSASTKGPSVFPLAPSSKSTSGGTAALGCLVKDYFPEPVTVSWNSGALTSGVHTFPAVLQSSGLYSLSSVVTVPSSSLGTQTYICNVNHKPSNTKVDKKVEPKSCDKTHTCPPCPAPELLGGPSVFLFPPKPKDTLMISRTPEVTCVVVDVSHEDPEVKFNWYVDGVEVHNAKTKPREEQYNSTYRVVSVLTVLHQDWLNGKEYKCKVSNMALPAPISKTISKAKGQPREPQVYTLPPSRDELTKNQVSLTCLVKGFYPSDIAVEWESNGQPENNYKTTPPVLDSDGSFFLYSKLTVDKSRWQQGNVFSCSVMHEALHNHYTQKSLSLSPGK

SEQ ID NO: 14 - protein, 465 aa, synthetic construct
MKHLWFFLLLVAAPRWVLSQVQLQESGPGLVKPSETLSLTCTVSGYSITSDYAWNWIRQFPGNKLEWMGYITYSGSTYYNPSLKSRVTISVDTSKNQFSLKLSSVTAADTATYYCVSGTYYFDYWGQGTTLTVSSASTKGPSVFPLAPSSKSTSGGTAALGCLVKDYFPEPVTVSWNSGALTSGVHTFPAVLQSSGLYSLSSVVTVPSSSLGTQTYICNVNHKPSNTKVDKKVEPKSCDKTHTCPPCPAPELLAGPSVFLFPPKPKDTLMISRTPEVTCVVVDVEFEDPEVKFNWYVDGVEVHNAKTKPREEQYNSTYRVVSVLTVLHQDWLNGKEYKCKVTNKALPAPEEKTISKAKGQPREPQVYTLPPSRDELTKNQVSLTCLVKGFYPSDIAVEWESNGQPENNYKTTPPVLDSDGSFFLYSKLTVDKSRWQQGNVFSCSVMHEALHNHYTQKSLSLSPGK

SEQ ID NO: 15 - protein, 465 aa, synthetic construct
MKHLWFFLLLVAAPRWVLSQVQLQESGPGLVKPSETLSLTCTVSGYSITSDYAWNWIRQFPGNKLEWMGYITYSGSTYYNPSLKSRVTISVETSKNQFSLKLSSVTAADTATYYCVSGTYYFDYWGQGTTLTVSSASTKGPSVFPLAPSSKSTSGGTAALGCLVKDYFPEPVTVSWNSGALTSGVHTFPAVLQSSGLYSLSSVVTVPSSSLGTQTYICNVNHKPSNTKVDKKVEPKSCDKTHTCPPCPAPELLGGPSVFLFPPKPKDTLMISRTPEVTCVVVDVSHEDPEVKFNWYVDGVEVHNAKTKPREEQYNSTYRVVSVLTVLHQDWLNGKEYKCKVSNKALPAPIEKTISKAKGQPREPQVYTLPPSRDELTKNQVSLTCLVKGFYPSDIAVEWESNGQPENNYKTTPPVLDSDGSFFLYSKLTVDKSRWQQGNVFSCSVMHEALHNHYTQKSLSLSPGK

SEQ ID NO: 16 - protein, 465 aa, synthetic construct
MKHLWFFLLLVAAPRWVLSQVQLQESGPGLVKPSETLSLTCTVSGYSITSDYAWNWIRQFPGNKLEWMGYITYSGSTYYNPSLKSRVTISVDTSKNQFSLKLSSVTAADTATYYCVSGTYYFDYWGQGTTLTVSSASTKGPSVFPLAPSSKSTSGGTAALGCLVKDYFPEPVTVSWNSGALTSGVHTFPAVLQSSGLYSLSSVVTVPSSSLGTQTYICNVNHKPSNTKVDKKVEPKSCDKTHTCPPCPAPEAAGGPSVFLFPPKPKDTLMISRTPEVTCVVVDVSHEDPEVKFNWYVDGVEVHNAKTKPREEQYNSTYRVVSVLTVLHQDWLNGKEYKCKVSNKALGAPIEKTISKAKGQPREPQVYTLPPSRDELTKNQVSLTCLVKGFYPSDIAVEWESNGQPENNYKTTPPVLDSDGSFFLYSKLTVDKSRWQQGNVFSCSVMHEALHNHYTQKSLSLSPGK

SEQ ID NO: 17 - protein, 244 aa, synthetic construct
MDMRVPAMDMRVPAQLLGLLLLWLPGARCDIQMTQSPSSLSASVGDRVTITCRASQSISRYLNWYQQKPGKAPKLLIYAASSLQSGVPSRFSGSGSGTDFTLTISSLQPEDFATYYCQQSYSTQRGAFGQGTKVEIKRTVAAPSVFIFPPSDEQLKSGTASVVCLLNNFYPREAKVQWKVDNALQSGNSQESVTEQDSKDSTYSLSSTLTLSKADYEKHKVYACEVTHQGLSSPVTKSFNRGEC

SEQ ID NO: 18 - protein, 482 aa, synthetic construct
MKHLWFFLLLVAAPRWVLSEVQLVESGGGVVQPGRSLRLSCAASGFTFSSYVMHWVRQAPGKGLEWVAVISEDGSNKYEADSVKGRFTISRDNSKNTLYLQMNSLRAEDTAVYYCARENVRPYYDFWRGYNSEYYYYGLDVWGQGTTVTVSSASTKGPSVFPLAPSSKSTSGGTAALGCLVKDYFPEPVTVSWNSGALTSGVHTFPAVLQSSGLYSLSSVVTVPSSSLGTQTYICNVNHKPSNTKVDKRVEPKSCDKTHTCPPCPAPELLGGPSVFLFPPKPKDTLMISRTPEVTCVVVDVSHEDPEVKFNWYVDGVEVHNAKTKPREEQYNSTYRVVSVLTVLHQDWLNGKEYKCKVSNKALPAPIEKTISKAKGQPREPQVYTLPPSREEMTKNQVSLTCLVKGFYPSDIAVEWESNGQPENNYKTTPPVLDSDGSFFLYSKLTVDKSRWQQGNVFSCSVMHEALHNHYTQKSLSLSPGK

SEQ ID NO: 19 - protein, 11 aa, synthetic construct
RASQSVSSDVA

SEQ ID NO: 20 - protein, 7 aa, synthetic construct
YASNRYS

SEQ ID NO: 21 - protein, 9 aa, synthetic construct
GQDYTSPRT

SEQ ID NO: 22 - protein, 6 aa, synthetic construct
SDYAWN

SEQ ID NO: 23 - protein, 16 aa, synthetic construct
YITYSGSTYYNPSLKS

SEQ ID NO: 24 - protein, 7 aa, synthetic construct
GTYYFDY

SEQ ID NO: 25 - protein, 9 aa, synthetic construct
QQDYTSPRT

SEQ ID NO: 26 - protein, 1156 aa, Homo sapiens
MSKLRMVLLEDSGSADFRRHFVNLSPFTITVVLLLSACFVTSSLGGTDKELRLVDGENKCSGRVEVKVQEEWGTVCNNGWSMEAVSVICNQLGCPTAIKAPGWANSSAGSGRIWMDHVSCRGNESALWDCKHDGWGKHSNCTHQQDAGVTCSDGSNLEMRLTRGGNMCSGRIEIKFQGRWGTVCDDNFNIDHASVICRQLECGSAVSFSGSSNFGEGSGPIWFDDLICNGNESALWNCKHQGWGKHNCDHAEDAGVICSKGADLSLRLVDGVTECSGRLEVRFQGEWGTICDDGWDSYDAAVACKQLGCPTAVTAIGRVNASKGFGHIWLDSVSCQGHEPAIWQCKHHEWGKHYCNHNEDAGVTCSDGSDLELRLRGGGSRCAGTVEVEIQRLLGKVCDRGWGLKEADVVCRQLGCGSALKTSYQVYSKIQATNTWLFLSSCNGNETSLWDCKNWQWGGLTCDHYEEAKITCSAHREPRLVGGDIPCSGRVEVKHGDTWGSICDSDFSLEAASVLCRELQCGTVVSILGGAHFGEGNGQIWAEEFQCEGHESHLSLCPVAPRPEGTCSHSRDVGVVCSRYTEIRLVNGKTPCEGRVELKTLGAWGSLCNSHWDIEDAHVLCQQLKCGVALSTPGGARFGKGNGQIWRHMFHCTGTEQHMGDCPVTALGASLCPSEQVASVICSGNQSQTLSSCNSSSLGPTRPTIPEESAVACIESGQLRLVNGGGRCAGRVEIYHEGSWGTICDDSWDLSDAHVVCRQLGCGEAINATGSAHFGEGTGPIWLDEMKCNGKESRIWQCHSHGWGQQNCRHKEDAGVICSEFMSLRLTSEASREACAGRLEVFYNGAWGTVGKSSMSETTVGVVCRQLGCADKGKINPASLDKAMSIPMWVDNVQCPKGPDTLWQCPSSPWEKRLASPSEETWITCDNKIRLQEGPTSCSGRVEIWHGGSWGTVCDDSWDLDDAQVVCQQLGCGPALKAFKEAEFGQGTGPIWLNEVKCKGNESSLWDCPARRWGHSECGHKEDAAVNCTDISVQKTPQKATTGRSSRQSSFIAVGILGVVLLAIFVALFFLTKKRRQRQRLAVSSRGENLVHQIQYREMNSCLNADDLDLMNSSENSHESADFSAAELISVSKFLPISGMEKEAILSHTEKENGNL